European Patent Application EP 4 112 083 A1, published January 4, 2023. Title: Antisense nucleic acids that induce exon 51 skipping. Applicant: Nippon Shinyaku Co., Ltd. National Center of Neurology and Psychiatry. The sequence listing filed with the application follows.

SEQUENCE LISTING (128 sequences)

SEQ ID NO: 1 - DNA, 27 bp, Artificial
  Synthetic Nucleic Acid
tcggtaagttctaagatggcatttcta

SEQ ID NO: 2 - DNA, 26 bp, Artificial
  Synthetic Nucleic Acid
tcggtaagttctaagatggcatttct

SEQ ID NO: 3 - DNA, 27 bp, Artificial
  Synthetic Nucleic Acid
tcggtaagttccatcaaggaagatggc

SEQ ID NO: 4 - DNA, 27 bp, Artificial
  Synthetic Nucleic Acid
cggtaagttccatcaaggaagatggca

SEQ ID NO: 5 - DNA, 28 bp, Artificial
  Synthetic Nucleic Acid
tcggtaagttctgtcaagatggcatttc

SEQ ID NO: 6 - DNA, 26 bp, Artificial
  Synthetic Nucleic Acid
tcggtaagttctgatggcatttctag

SEQ ID NO: 7 - DNA, 26 bp, Artificial
  Synthetic Nucleic Acid
ccagtcggtaagtgatggcatttcta

SEQ ID NO: 8 - DNA, 26 bp, Artificial
  Synthetic Nucleic Acid
tcggtaagttctgagatggcatttct

SEQ ID NO: 9 - DNA, 26 bp, Artificial
  Synthetic Nucleic Acid
tcggtaagttctgtaagatggcattt

SEQ ID NO: 10 - DNA, 26 bp, Artificial
  Synthetic Nucleic Acid
cggtaagttctgtcaagatggcattt

SEQ ID NO: 11 - DNA, 25 bp, Artificial
  Synthetic Nucleic Acid
tcggtaagttctagatggcatttct

SEQ ID NO: 12 - DNA, 26 bp, Artificial
  Synthetic Nucleic Acid
tcggtaagttctgtatggcatttcta

SEQ ID NO: 13 - DNA, 26 bp, Artificial
  Synthetic Nucleic Acid
tcggtaagttctggatggcatttcta

SEQ ID NO: 14 - DNA, 26 bp, Artificial
  Synthetic Nucleic Acid
tcggtaagttctgtgatggcatttct

SEQ ID NO: 15 - DNA, 25 bp, Artificial
  Synthetic Nucleic Acid
tcggtaagttctggatggcatttct

SEQ ID NO: 16 - DNA, 26 bp, Artificial
  Synthetic Nucleic Acid
tcggtaagttctgtagatggcatttc

SEQ ID NO: 17 - DNA, 25 bp, Artificial
  Synthetic Nucleic Acid
tcggtaagttctgaagatggcattt

SEQ ID NO: 18 - DNA, 25 bp, Artificial
  Synthetic Nucleic Acid
gtcggtaagttctagatggcatttc

SEQ ID NO: 19 - DNA, 23 bp, Artificial
  Synthetic Nucleic Acid
tcggtaagttctgatggcatttc

SEQ ID NO: 20 - DNA, 25 bp, Artificial
  Synthetic Nucleic Acid
cggtaagttctgagatggcatttct

SEQ ID NO: 21 - DNA, 25 bp, Artificial
  Synthetic Nucleic Acid
tcggtaagttctgagatggcatttc

SEQ ID NO: 22 - DNA, 24 bp, Artificial
  Synthetic Nucleic Acid
tcggtaagttctggaagatggcat

SEQ ID NO: 23 - DNA, 25 bp, Artificial
  Synthetic Nucleic Acid
cggtaagttctgtagatggcatttc

SEQ ID NO: 24 - DNA, 23 bp, Artificial
  Synthetic Nucleic Acid
cggtaagttctgagatggcattt

SEQ ID NO: 25 - DNA, 23 bp, Artificial
  Synthetic Nucleic Acid
cggtaagttctggatggcatttc

SEQ ID NO: 26 - DNA, 23 bp, Artificial
  Synthetic Nucleic Acid
cggtaagttctgatggcatttct

SEQ ID NO: 27 - DNA, 24 bp, Artificial
  Synthetic Nucleic Acid
cggtaagttctgtatggcatttct

SEQ ID NO: 28 - DNA, 22 bp, Artificial
  Synthetic Nucleic Acid
cggtaagttctgatggcatttc

SEQ ID NO: 29 - DNA, 25 bp, Artificial
  Synthetic Nucleic Acid
cagtcggtaagttcatggcatttct

SEQ ID NO: 30 - DNA, 25 bp, Artificial
  Synthetic Nucleic Acid
cggtaagttctgtccgaagatggca

SEQ ID NO: 31 - DNA, 25 bp, Artificial
  Synthetic Nucleic Acid
cggtaagttctgtgatggcatttct

SEQ ID NO: 32 - DNA, 25 bp, Artificial
  Synthetic Nucleic Acid
cggtaagttctgtcatggcatttct

SEQ ID NO: 33 - DNA, 27 bp, Artificial
  Synthetic Nucleic Acid
cagtcggtaagttccatcaaggaagat

SEQ ID NO: 34 - DNA, 27 bp, Artificial
  Synthetic Nucleic Acid
tcggtaagttctatcaaggaagatggc

SEQ ID NO: 35 - DNA, 27 bp, Artificial
  Synthetic Nucleic Acid
cagtcggtaagttgaagatggcatttc

SEQ ID NO: 36 - DNA, 28 bp, Artificial
  Synthetic Nucleic Acid
aaagccagtcggtaacatcaaggaagat

SEQ ID NO: 37 - DNA, 30 bp, Artificial
  Synthetic Nucleic Acid
cagtcggtaagttctatcaaggaagatggc

SEQ ID NO: 38 - DNA, 30 bp, Artificial
  Synthetic Nucleic Acid
agccagtcggtaagtaacatcaaggaagat

SEQ ID NO: 39 - DNA, 27 bp, Artificial
  Synthetic Nucleic Acid
aaagccagtcggaacatcaaggaagat

SEQ ID NO: 40 - DNA, 28 bp, Artificial
  Synthetic Nucleic Acid
cagtcggtaagttcgaagatggcatttc

SEQ ID NO: 41 - DNA, 27 bp, Artificial
  Synthetic Nucleic Acid
aaagccagtcggtacatcaaggaagat

SEQ ID NO: 42 - DNA, 27 bp, Artificial
  Synthetic Nucleic Acid
tcggtaagttctgtcaagatggcattt

SEQ ID NO: 43 - DNA, 27 bp, Artificial
  Synthetic Nucleic Acid
ccagtcggtaagtaagatggcatttct

SEQ ID NO: 44 - DNA, 27 bp, Artificial
  Synthetic Nucleic Acid
tcggtaagttctgtcatcaaggaagat

SEQ ID NO: 45 - DNA, 27 bp, Artificial
  Synthetic Nucleic Acid
tcggtaagttctcaaggaagatggcat

SEQ ID NO: 46 - DNA, 28 bp, Artificial
  Synthetic Nucleic Acid
gtcggtaagttcttcaaggaagatggca

SEQ ID NO: 47 - DNA, 28 bp, Artificial
  Synthetic Nucleic Acid
tcggtaagttctatcaaggaagatggca

SEQ ID NO: 48 - DNA, 27 bp, Artificial
  Synthetic Nucleic Acid
cagtcggtaagttcacatcaaggaaga

SEQ ID NO: 49 - DNA, 27 bp, Artificial
  Synthetic Nucleic Acid
cggtaagttctcaacatcaaggaagat

SEQ ID NO: 50 - DNA, 26 bp, Artificial
  Synthetic Nucleic Acid
gtcggtaagttctcatcaaggaagat

SEQ ID NO: 51 - DNA, 27 bp, Artificial
  Synthetic Nucleic Acid
ccagtcggtaagaacatcaaggaagat

SEQ ID NO: 52 - DNA, 28 bp, Artificial
  Synthetic Nucleic Acid
aagccagtcggtaaacatcaaggaagat

SEQ ID NO: 53 - DNA, 27 bp, Artificial
  Synthetic Nucleic Acid
tcggtaagttctgcatcaaggaagatg

SEQ ID NO: 54 - DNA, 27 bp, Artificial
  Synthetic Nucleic Acid
tcggtaagttctaaggaagatggcatt

SEQ ID NO: 55 - DNA, 29 bp, Artificial
  Synthetic Nucleic Acid
tcggtaagttcttcaaggaagatggcatt

SEQ ID NO: 56 - DNA, 28 bp, Artificial
  Synthetic Nucleic Acid
agaaagccagtccatcaaggaagatggc

SEQ ID NO: 57 - DNA, 28 bp, Artificial
  Synthetic Nucleic Acid
agtcggtaagttcaacatcaaggaagat

SEQ ID NO: 58 - DNA, 29 bp, Artificial
  Synthetic Nucleic Acid
ccagtcggtaagttaacatcaaggaagat

SEQ ID NO: 59 - DNA, 29 bp, Artificial
  Synthetic Nucleic Acid
agtcggtaagttctaacatcaaggaagat

SEQ ID NO: 60 - DNA, 28 bp, Artificial
  Synthetic Nucleic Acid
ccagtcggtaagtaacatcaaggaagat

SEQ ID NO: 61 - DNA, 28 bp, Artificial
  Synthetic Nucleic Acid
tcggtaagttctcatcaaggaagatggc

SEQ ID NO: 62 - DNA, 28 bp, Artificial
  Synthetic Nucleic Acid
agccagtcggtaaaacatcaaggaagat

SEQ ID NO: 63 - DNA, 30 bp, Artificial
  Synthetic Nucleic Acid
tcggtaagttctgtcctctgagtaggagct

SEQ ID NO: 64 - DNA, 27 bp, Artificial
  Synthetic Nucleic Acid
taacagtctgagtcggtaagttctgtc

SEQ ID NO: 65 - DNA, 27 bp, Artificial
  Synthetic Nucleic Acid
cggtaagttctgtcagtaacagtctga

SEQ ID NO: 66 - DNA, 27 bp, Artificial
  Synthetic Nucleic Acid
cggtaagttctgtcacagtctgagtag

SEQ ID NO: 67 - DNA, 27 bp, Artificial
  Synthetic Nucleic Acid
cggtaagttctgtccaacagtctgagt

SEQ ID NO: 68 - DNA, 26 bp, Artificial
  Synthetic Nucleic Acid
tcggtaagttctgtccagtctgagta

SEQ ID NO: 69 - DNA, 26 bp, Artificial
  Synthetic Nucleic Acid
tcggtaagttctgtacagtctgagta

SEQ ID NO: 70 - DNA, 26 bp, Artificial
  Synthetic Nucleic Acid
tcggtaagttctgtcacagtctgagt

SEQ ID NO: 71 - DNA, 27 bp, Artificial
  Synthetic Nucleic Acid
tcggtaagttctgtaacagtctgagta

SEQ ID NO: 72 - DNA, 27 bp, Artificial
  Synthetic Nucleic Acid
tcggtaagttctgtcaacagtctgagt

SEQ ID NO: 73 - DNA, 27 bp, Artificial
  Synthetic Nucleic Acid
tcggtaagttctgttaacagtctgagt

SEQ ID NO: 74 - DNA, 26 bp, Artificial
  Synthetic Nucleic Acid
tcggtaagttctgtctctgagtagga

SEQ ID NO: 75 - DNA, 25 bp, Artificial
  Synthetic Nucleic Acid
tcggtaagttctgtcctgagtagga

SEQ ID NO: 76 - DNA, 26 bp, Artificial
  Synthetic Nucleic Acid
tcggtaagttctgtctgagtaggagc

SEQ ID NO: 77 - DNA, 25 bp, Artificial
  Synthetic Nucleic Acid
cggtaagttctgtccagtctgagta

SEQ ID NO: 78 - DNA, 22 bp, Artificial
  Synthetic Nucleic Acid
tcggtaagttctgtctgagtag

SEQ ID NO: 79 - DNA, 25 bp, Artificial
  Synthetic Nucleic Acid
tcggtaagttctgtcgtaggagcta

SEQ ID NO: 80 - DNA, 25 bp, Artificial
  Synthetic Nucleic Acid
tcggtaagttctgtgagtaggagct

SEQ ID NO: 81 - DNA, 25 bp, Artificial
  Synthetic Nucleic Acid
cggtaagttctgtccctgagtagga

SEQ ID NO: 82 - DNA, 27 bp, Artificial
  Synthetic Nucleic Acid
taagttctgtccgtctgagtaggagct

SEQ ID NO: 83 - DNA, 28 bp, Artificial
  Synthetic Nucleic Acid
cggtaagttctgtcgtaggagctaaaat

SEQ ID NO: 84 - DNA, 28 bp, Artificial
  Synthetic Nucleic Acid
tctgtccaagcccgctgagtaggagcta

SEQ ID NO: 85 - DNA, 27 bp, Artificial
  Synthetic Nucleic Acid
cggtaagttctgtctaacagtctgagt

SEQ ID NO: 86 - DNA, 28 bp, Artificial
  Synthetic Nucleic Acid
agttctgtccaacagtctgagtaggagc

SEQ ID NO: 87 - DNA, 27 bp, Artificial
  Synthetic Nucleic Acid
taagttctgtccaatctgagtaggagc

SEQ ID NO: 88 - DNA, 26 bp, Artificial
  Synthetic Nucleic Acid
cggtaagttctgtcaacagtctgagt

SEQ ID NO: 89 - DNA, 26 bp, Artificial
  Synthetic Nucleic Acid
tcggtaagttctgtaacagtctgagt

SEQ ID NO: 90 - DNA, 30 bp, Artificial
  Synthetic Nucleic Acid
cggtaagttctgtcctcaaggaagatggca

SEQ ID NO: 91 - DNA, 28 bp, Artificial
  Synthetic Nucleic Acid
tcggtaagttctgtcgaagatggcattt

SEQ ID NO: 92 - DNA, 27 bp, Artificial
  Synthetic Nucleic Acid
cggtaagttctgtcaagatggcatttc

SEQ ID NO: 93 - DNA, 28 bp, Artificial
  Synthetic Nucleic Acid
cggtaagttctgtccgaagatggcattt

SEQ ID NO: 94 - DNA, 30 bp, Artificial
  Synthetic Nucleic Acid
ctccaacatcaaggaagatggcatttctag

SEQ ID NO: 95 - DNA, 20 bp, Artificial
  Synthetic Nucleic Acid
ctgagtggaaggcggtaaac

SEQ ID NO: 96 - DNA, 20 bp, Artificial
  Synthetic Nucleic Acid
gaagtttcagggccaagtca

SEQ ID NO: 97 - DNA, 30 bp, Artificial
  Synthetic Nucleic Acid
ctcataccttctgcttcaaggaagatggca

SEQ ID NO: 98 - DNA, 30 bp, Artificial; identical to SEQ ID NO: 94
  Synthetic Nucleic Acid

SEQ ID NO: 99 - DNA, 21 bp, Artificial
  Synthetic Nucleic Acid
aacatcaaggaagatggcatt

SEQ ID NO: 100 - DNA, 21 bp, Artificial
  Synthetic Nucleic Acid
tccaacatcaaggaagatggc

SEQ ID NO: 101 - DNA, 21 bp, Artificial
  Synthetic Nucleic Acid
acctccaacatcaaggaagat

SEQ ID NO: 102 - RNA, 21 nt, Artificial
  Synthetic Nucleic Acid
gaguaacagucugaguaggag

SEQ ID NO: 103 - RNA, 21 nt, Artificial
  Synthetic Nucleic Acid
ugugucaccagaguaacaguc

SEQ ID NO: 104 - RNA, 21 nt, Artificial
  Synthetic Nucleic Acid
aaccacagguugugucaccag

SEQ ID NO: 105 - RNA, 21 nt, Artificial
  Synthetic Nucleic Acid
uuuccuuaguaaccacagguu

SEQ ID NO: 106 - RNA, 21 nt, Artificial
  Synthetic Nucleic Acid
gagauggcaguuuccuuagua

SEQ ID NO: 107 - RNA, 21 nt, Artificial
  Synthetic Nucleic Acid
uucuaguuuggagauggcagu

SEQ ID NO: 108 - RNA, 21 nt, Artificial
  Synthetic Nucleic Acid
aagauggcauuucuaguuugg

SEQ ID NO: 109 - RNA, 21 nt, Artificial
  Synthetic Nucleic Acid
aacaucaaggaagauggcauu

SEQ ID NO: 110 - RNA, 21 nt, Artificial
  Synthetic Nucleic Acid
agguaccuccaacaucaagga

SEQ ID NO: 111 - RNA, 21 nt, Artificial
  Synthetic Nucleic Acid
cugccagagcagguaccucca

SEQ ID NO: 112 - RNA, 21 nt, Artificial
  Synthetic Nucleic Acid
cgguugaaaucugccagagca

SEQ ID NO: 113 - RNA, 21 nt, Artificial
  Synthetic Nucleic Acid
uguccaagcccgguugaaauc

SEQ ID NO: 114 - RNA, 21 nt, Artificial
  Synthetic Nucleic Acid
cgguaaguucuguccaagccc

SEQ ID NO: 115 - RNA, 21 nt, Artificial
  Synthetic Nucleic Acid
gaaagccagucgguaaguucu

SEQ ID NO: 116 - RNA, 21 nt, Artificial
  Synthetic Nucleic Acid
aucaagcagagaaagccaguc

SEQ ID NO: 117 - RNA, 21 nt, Artificial
  Synthetic Nucleic Acid
uuauaacuugaucaagcagag

SEQ ID NO: 118 - RNA, 21 nt, Artificial
  Synthetic Nucleic Acid
cucugugauuuuauaacuuga

SEQ ID NO: 119 - RNA, 21 nt, Artificial
  Synthetic Nucleic Acid
caccaucacccucugugauuu

SEQ ID NO: 120 - RNA, 21 nt, Artificial
  Synthetic Nucleic Acid
caaggucacccaccaucaccc

SEQ ID NO: 121 - RNA, 21 nt, Artificial
  Synthetic Nucleic Acid
uugauauccucaaggucaccc

SEQ ID NO: 122 - RNA, 21 nt, Artificial
  Synthetic Nucleic Acid
gaucaucucguugauauccuc

SEQ ID NO: 123 - RNA, 21 nt, Artificial
  Synthetic Nucleic Acid
ucugcuugaugaucaucucgu

SEQ ID NO: 124 - RNA, 21 nt, Artificial
  Synthetic Nucleic Acid
ggcauuucuaguuuggagaug

SEQ ID NO: 125 - RNA, 21 nt, Artificial
  Synthetic Nucleic Acid
caaggaagauggcauuucuag

SEQ ID NO: 126 - RNA, 21 nt, Artificial
  Synthetic Nucleic Acid
ccuccaacaucaaggaagaug

SEQ ID NO: 127 - DNA, 233 bp, Homo sapiens
ctcctactcagactgttactctggtgacacaacctgtggttactaaggaaactgccatctccaaactagaaatgccatcttccttgatgttggaggtacctgctctggcagatttcaaccgggcttggacagaacttaccgactggctttctctgcttgatcaagttataaaatcacagagggtgatggtgggtgaccttgaggatatcaacgagatgatcatcaagcagaag

SEQ ID NO: 128 - DNA, 251 bp, Homo sapiens
aaacccaaaatattttagctcctactcagactgttactctggtgacacaacctgtggttactaaggaaactgccatctccaaactagaaatgccatcttccttgatgttggaggtacctgctctggcagatttcaaccgggcttggacagaacttaccgactggctttctctgcttgatcaagttataaaatcacagagggtgatggtgggtgaccttgaggatatcaacgagatgatcatcaagcagaag